European Patent Application EP 4 585 618 A1, published July 16, 2025. Title: ANTI-ILT4 ANTIBODY AND PHARMACEUTICAL USE THEREOF. Applicant: JIANGSU HENGRUI PHARMACEUTICALS CO., LTD. Application WO. The sequence listing filed with the application follows.

SEQUENCE LISTING (273 sequences)

SEQ ID NO: 1 - protein, 672 aa, synthetic construct
  CHAIN 1..672: note = ILT4-Fc
QTGTIPKPTLWAEPDSVITQGSPVTLSCQGSLEAQEYRLYREKKSASWITRIRPELVKNGQFHIPSITWEHTGRYGCQYYSRARWSELSDPLVLVMTGAYPKPTLSAQPSPVVTSGGRVTLQCESQVAFGGFILCKEGEEEHPQCLNSQPHARGSSRAIFSVGPVSPNRRWSHRCYGYDLNSPYVWSSPSDLLELLVPGVSKKPSLSVQPGPVVAPGESLTLQCVSDVGYDRFVLYKEGERDLRQLPGRQPQAGLSQANFTLGPVSRSYGGQYRCYGAHNLSSECSAPSDPLDILITGQIRGTPFISVQPGPTVASGENVTLLCQSWRQFHTFLLTKAGAADAPLRLRSIHEYPKYQAEFPMSPVTSAHAGTYRCYGSLNSDPYLLSHPSEPLELVVSGPSMGSSPPPTGPISTPAGPEDQPLTPTGSDPQSGLGRHLGVEPKSSDKTHTCPPCPAPELLGGPSVFLFPPKPKDTLMISRTPEVTCVVVDVSHEDPEVKFNWYVDGVEVHNAKTKPREEQYNSTYRVVSVLTVLHQDWLNGKEYKCKVSNKALPAPIEKTISKAKGQPREPQVYTLPPSRDELTKNQVSLTCLVKGFYPSDIAVEWESNGQPENNYKTTPPVLDSDGSFFLYSKLTVDKSRWQQGNVFSCSVMHEALHNHYTQKSLSLSPGK

SEQ ID NO: 2 - protein, 446 aa, synthetic construct
  CHAIN 1..446: note = ILT4-His
QTGTIPKPTLWAEPDSVITQGSPVTLSCQGSLEAQEYRLYREKKSASWITRIRPELVKNGQFHIPSITWEHTGRYGCQYYSRARWSELSDPLVLVMTGAYPKPTLSAQPSPVVTSGGRVTLQCESQVAFGGFILCKEGEEEHPQCLNSQPHARGSSRAIFSVGPVSPNRRWSHRCYGYDLNSPYVWSSPSDLLELLVPGVSKKPSLSVQPGPVVAPGESLTLQCVSDVGYDRFVLYKEGERDLRQLPGRQPQAGLSQANFTLGPVSRSYGGQYRCYGAHNLSSECSAPSDPLDILITGQIRGTPFISVQPGPTVASGENVTLLCQSWRQFHTFLLTKAGAADAPLRLRSIHEYPKYQAEFPMSPVTSAHAGTYRCYGSLNSDPYLLSHPSEPLELVVSGPSMGSSPPPTGPISTPAGPEDQPLTPTGSDPQSGLGRHLGVHHHHHH

SEQ ID NO: 3 - protein, 598 aa, synthetic construct
  CHAIN 1..598: note = CHO-S/ILT4
MTPIVTVLICLGLSLGPRTHVQTGTIPKPTLWAEPDSVITQGSPVTLSCQGSLEAQEYRLYREKKSASWITRIRPELVKNGQFHIPSITWEHTGRYGCQYYSRARWSELSDPLVLVMTGAYPKPTLSAQPSPVVTSGGRVTLQCESQVAFGGFILCKEGEEEHPQCLNSQPHARGSSRAIFSVGPVSPNRRWSHRCYGYDLNSPYVWSSPSDLLELLVPGVSKKPSLSVQPGPVVAPGESLTLQCVSDVGYDRFVLYKEGERDLRQLPGRQPQAGLSQANFTLGPVSRSYGGQYRCYGAHNLSSECSAPSDPLDILITGQIRGTPFISVQPGPTVASGENVTLLCQSWRQFHTFLLTKAGAADAPLRLRSIHEYPKYQAEFPMSPVTSAHAGTYRCYGSLNSDPYLLSHPSEPLELVVSGPSMGSSPPPTGPISTPAGPEDQPLTPTGSDPQSGLGRHLGVVIGILVAVVLLLLLLLLLFLILRHRRQGKHWTSTQRKADFQHPAGAVGPEPTDRGLQWRSSPAADAQEENLYAAVKDTQPEDGVEMDTRAAASEAPQDVTYAQLHSLTLRRKATEPPPSQEREPPAEPSIYATLAIH

SEQ ID NO: 4 - protein, 117 aa, Mus musculus
  source 1..117: note = HCVR
  REGION 1..117: note = M P1-B4 HCVR
QVQLKQSGPGLVQPSQSLSITCTVSSFSLTNYGVHWVRQSPGKGLEWLGVIWTGGSTDYNAAFISRLSIIRDNSKSQVFFKMNSLQADDTAMYYCAITTVVTAMDYWGQGTSVTVSS

SEQ ID NO: 5 - protein, 107 aa, Mus musculus
  source 1..107: note = LCVR
  REGION 1..107: note = M P1-B4 LCVR
DIVMTQSHKFMSTSVGDRVSITCKASQDVNIAVVWYQQKPGQSPKLLIYAASYRYTGVPDRFTGSGSGTDFTFTISSVQAEDLAVYYCQQHYSSPYTFGGGTKLEIK

SEQ ID NO: 6 - protein, 117 aa, Mus musculus
  source 1..117: note = HCVR
  REGION 1..117: note = M P1-B9 HCVR
QVQLKQSGPGLVQPSQSLSITCTVSGFSLTSYGVHWVRQSPGKGLEWLGVIWSGGNTDYNAAFMSRLRINKDNSKSQVFFKMNSLQGSDTAIYYCATPYDVVPFAYWGQGTLVTVSS

SEQ ID NO: 7 - protein, 107 aa, Mus musculus
  source 1..107: note = LCVR
  REGION 1..107: note = M P1-B9 LCVR
DIVMTQSHKFMSTSVGDRVSITCKASQDVNIAVAWYQQKPGLSPKLLIYSASYRYTGVPGRFTGSGSGTDFTFTISSVKAEDLAVYYCQQHYSIPFTFGAGTKLEIK

SEQ ID NO: 8 - protein, 115 aa, Mus musculus
  source 1..115: note = HCVR
  REGION 1..115: note = M P1-D10 HCVR
QVQLKQSGPGLVQPSQSLSITCTVSGFSLTTYGVHWVRQSPGKGLEWLGVIWSGGNTDSNAAFISRLSISKDNSKSQVFFKMNNLQADDTAIYYCARYSYAMDYWGQGTSVTVSS

SEQ ID NO: 9 - protein, 107 aa, Mus musculus
  source 1..107: note = LCVR
  REGION 1..107: note = M P1-D10 LCVR
DIVMTQSHKFMSTSVGDRVSITCKASQDVSNGVAWYQQKPGQSPKVLIYAASYRYTGVPDRFTGSGSGTDFTFTIGSVQAEDLALYYCQQHYSTPFTFGSGTMLEIK

SEQ ID NO: 10 - protein, 122 aa, Mus musculus
  source 1..122: note = HCVR
  REGION 1..122: note = M P2-E8 HCVR
EVQLLESGGGLVKPGGSLKLSCAASGFTFSDYGIHWVRQAPEKGLEWVAYISSGSSIINYADTVKGRFTISRDNAKNTLLLQMTSLRSEDTAMYYCARGPNYYGSSYLLVYWGQGTLVTVSS

SEQ ID NO: 11 - protein, 107 aa, Mus musculus
  source 1..107: note = LCVR
  REGION 1..107: note = M P2-E8 LCVR
DIVMTQSHKFMSTSVGDRVSITCKASQDVNIAVAWYQQRPGQSPKLLIYSASYRYTGVPDRFTGSGSGTDFTFTISSVQAEDLAVYYCQQHYNIPWTFGGGTKLEIK

SEQ ID NO: 12 - protein, 120 aa, Mus musculus
  REGION 1..120: note = M P2-C10 HCVR
QVQLQQPGAELVKPGASVKLSCKASGYTFTSYWMHWVKQRPGQGLEWIGVIHPNSDTTNYNEKFKNKATLTVDKSSSTAYMQLSSLTSEDSAVYYCATRYDYAYYAMDYWGQGTSVTVSS

SEQ ID NO: 13 - protein, 107 aa, Mus musculus
  REGION 1..107: note = M P2-C10 LCVR
DIVMTQSHKFMSTSVGDRVSITCKASQDVTTAVAWYQQKPGQSPKLLIYSASYRYTGVPDRFTGSGSGTDFTFTISSVQAEDLAVYHCQQHYSTSPTFGGGTMLEIK

SEQ ID NO: 14 - protein, 120 aa, Mus musculus
  REGION 1..120: note = M P2-F4 HCVR
EVQLVESGGGLVKPGGSLKLSCAASGFTFSDYGMHWVRQAPEKGLEWVAYISSGSRIIYYADTVKGRFTISRDNAKNTLFLQMTSLRSEDTAMYSCARFYNYAHYTMDYWGQGTSVTVSS

SEQ ID NO: 15 - protein, 107 aa, Mus musculus
  REGION 1..107: note = M P2-F4 LCVR
DIVMTQSHKFMSTSVGDRVSITCKASQDVSTAVAWYQQKPGQSPKLLIYSASYRYTGVPDRFTGSGSGTDFTFTISSVQAEDLTLYYCQHHYSTPPTFGGGTKLEIK

SEQ ID NO: 16 - protein, 117 aa, Mus musculus
  REGION 1..117: note = M P2-B3 HCVR
QVQLKQSGPGLVQPSQSLSITCTVSGFSLTNYGVHWFRQSPGKGLEWLGMIWSGGNTDYNAAFTSRLIITKDNSKSQVFFKMNSMQADDTAIYYCARGDYGSSSAYWGQGTLVTVSS

SEQ ID NO: 17 - protein, 107 aa, Mus musculus
  REGION 1..107: note = M P2-B3 LCVR
DIVMTQSHKFMSTSVGDRVSITCKASQDVSIAVAWYQQKPGQSPKLLIYSASYRYTGVPDRFTGSGSGTDFTFTISSVQAEDLAVYYCQQHYSNTLTFGAGTKLEIK

SEQ ID NO: 18 - protein, 121 aa, Mus musculus
  REGION 1..121: note = M P2-E7 HCVR
QVQLQQPGTELVKPGASVKLSCKASGYTFTSYWMHWVKQSPGQGLEWIGNINPSNGGPNYNENFKTKATLTVDKSSSTAYMQLNSLTSEDSAVYYCAGGDYYGGSYLFAYWGQGTLVTVSS

SEQ ID NO: 19 - protein, 107 aa, Mus musculus
  REGION 1..107: note = M P2-E7 LCVR
DTVMTQSHKFMSTSVGDRVSVTCKASQDVNIAVAWYQQKPGQSPKLLIYSSSYRYTGVPDRFTGSGSETDFTFTISSVQAEDLAVYYCQQHYTFPYTFGGGTKLEIK

SEQ ID NO: 20 - protein, 121 aa, Mus musculus
  REGION 1..121: note = M P2-G4 HCVR
EVQLQQSGPELVKPGASVKMSCKASGYTFTDYNMHWVKQSHGKSLEWIGYINPNNGGTTYNQKFKGKATLTVNKSSSTAYMELRSLTSEDSAVYYCASSEYYGSTFLFAYWGQGTLVTVSS

SEQ ID NO: 21 - protein, 107 aa, Mus musculus
  REGION 1..107: note = M P2-G4 LCVR
DIVMTQSHKFMSTSVGDRVGITCKASQDVSIAVAWYQQKPGQSPKLLIYSASYRYTGVPDRFTGSGSGTDFTFTISSVQAEDLAAYYCQQHYSTPWTFGGGTKLEIK

SEQ ID NO: 22 - protein, 116 aa, Mus musculus
  REGION 1..116: note = M P2-C4 HCVR
QVQLKESGPGLVAPSQSLSITCTVSGFSLSTYAIGWVRQPPGKGLEWLGVIWTGGGTSYNSALKSRLSISKDNSKSQVFLKMNSLQTDDTARYYCARGDYGPFAYWGQGTLVTVSS

SEQ ID NO: 23 - protein, 107 aa, Mus musculus
  REGION 1..107: note = M P2-C4 LCVR
DIVMTQSHKFMSTSLGDRVSISCKASQDVSIAVAWYQQKAGQSPKLLIYSASYRHTGVPDRFTGSGSGTDFTFTISSVQAEDLAVYYCQQHYSTPFTFGSGTKLEIK

SEQ ID NO: 24 - protein, 121 aa, Mus musculus
  REGION 1..121: note = M P2-E11 HCVR
QVQLQQSGPELVKPGASVKISCKASAYTFTDYYINWVKQRPGQGLEWIGWIFPGSGSTYYNEKFKGKATLTVDKSSSTAYMLVSSLTSEDSAVYFCARSGTLVAPYAMDYWGQGTSVTVSS

SEQ ID NO: 25 - protein, 107 aa, Mus musculus
  REGION 1..107: note = M P2-E11 LCVR
SIVMTQTPKFLLVSAGDRVTITCKASQSVSNDVAWYQQKPGQSPKLLIYYTSNRYTGVPDRFTGSGYGTDFTFTISTVQAEDLAVYFCQQDYSFPLTFGAGTKLEIK

SEQ ID NO: 26 - protein, 122 aa, Mus musculus
  REGION 1..122: note = M P1-F7 HCVR
DVQLQESGPGLVKPSQSLSLTCSVTGYSITSGYYWNWIRQFPGNKLEWMGYISYDGNNYYNPSLKNRISVTRDTSKNQFFLKLNSVTSEDTATYYCAREDGSYSDYDGFAYWGQGTLVTVSS

SEQ ID NO: 27 - protein, 107 aa, Mus musculus
  REGION 1..107: note = M P1-F7 LCVR
DIQMTQSPASLSVSVGETVTITCRANENIYSNLAWYQQKQGKSPQLLVYAATNLADGVSSRFSGSGSGTQYSLRINSLQSEDFGSYYCQQFWGTPYTFGGGTKLEIK

SEQ ID NO: 28 - protein, 124 aa, Mus musculus
  REGION 1..124: note = M P2-E3 HCVR
EVQLQQSGPELVKPGASVKISCKASGYTFTDYYMNWVKQSHGKSLEWIGDINPNNGGTSYNQKFKGKATLTVDKSSSTAYMELRSLTSEDSTVYYCARGGVTTVVATYWYFDVWGTGTTVTVSS

SEQ ID NO: 29 - protein, 107 aa, Mus musculus
  REGION 1..107: note = M P2-E3 LCVR
DIQMTQSPASLSVSVGETVTITCRASENIYSNLAWYQQKQGKSPQLLVYAATNVADGVPSRFSGGGSGTQYSLKINSLQSEDFGSYYCQQFWDTPFTFGSGTKLEIK

SEQ ID NO: 30 - protein, 122 aa, Mus musculus
  REGION 1..122: note = M P2-F10 HCVR
DVQLQESGPGLVKPSQSLSLTCSVTGYSIASGYYWNWIRQFPGNKLEWMGYITYDGSNNYNPSLKNRISITRDTSKNQFFLKLNSVTTEDTATYYCAREYSYGSTLSWFAYWGQGTLVTVSS

SEQ ID NO: 31 - protein, 107 aa, Mus musculus
  REGION 1..107: note = M P2-F10 LCVR
DIQMTQSPASLSISVGETVTITCRASENIYSNLAWYQQKQGKSPQLLVYAATNLADGVPSRFSGSGSGTQYSLKINSLQSEDFGSYYCQHFWDTPYTFGGGTKLEIK

SEQ ID NO: 32 - protein, 123 aa, Mus musculus
  REGION 1..123: note = M P2-G9 HCVR
DVQLQESGPGLVKPSQSLSLACSVTGSSITSGYYWNWIRQFPGNKLEWMGYLSYDGSNNYNPSLKNRISITRDTSKSQFFLKLNSVTPEDTATYYCAREGAHYSGTLSWFAYWGQGTLVTVSS

SEQ ID NO: 33 - protein, 107 aa, Mus musculus
  REGION 1..107: note = M P2-G9 LCVR
DIQMTQSPASLSVSVGETVTITCRASENIYSNLAWYQQKQGKSPQLLVYAATNLADGVPSRFSGSGSGTQYSLKINSLQSEDFGSYYCQHFWDTPYTFGGGTKLEIK

SEQ ID NO: 34 - protein, 122 aa, Mus musculus
  REGION 1..122: note = M P1-C4 HCVR
QVQLKQSGAELVRPGASVKLSCKASGYSFTDYYINWVKQRPGQGLEWIARIYPGNDNTYYNEKFKDKATLTADSSSSTAYMQLSSLTSEDSAVYFCTRSQDGYYEENAMDYWGQGTSVTVSS

SEQ ID NO: 35 - protein, 107 aa, Mus musculus
  REGION 1..107: note = M P1-C4 LCVR
DIQMTQSPASLSVSVGETVTITCRASENIYSNLAWYQQRQGKSPQLLVYAATNLADGVPFRFSGSGSGTQYSLKINSLQSEDFGSYYCQQFWGSPHTFGGGTKLEIK

SEQ ID NO: 36 - protein, 122 aa, Mus musculus
  REGION 1..122: note = M P1-G7 HCVR
DVQLQESGPGLVKPSQSLSLTCSVTGYSITSGYYWNWIRQFPENKLEWMGYISYDGGNNYNPFLKNRISITRDTSKNQFFLNLNSVTIEDTATYYCAREGGSSWEYYGMDYWGQGTSVTVSS

SEQ ID NO: 37 - protein, 107 aa, Mus musculus
  REGION 1..107: note = M P1-G7 LCVR
DIQMTQSPASLSVSVGETVTITCRASENIYRNLAWYQQKQGHSPQLLLYAATNLADGVPSRFSGSGSGTQYSLKINSLQSEDFGSYYCQQFWGSPYTFGGGTKLEIK

SEQ ID NO: 38 - protein, 124 aa, Mus musculus
  REGION 1..124: note = M P2-C7 HCVR
EVQLQQSGPELVKPGTSVKMSCKASGYTFTDYSMHWVRQSHGKSLEWIGYFNPNNGDTIYNQKFKGKATLTVNKSSSTAYMELRSLTSDDSAVYYCAREDSVSTNAWDGALDYWGQGTSVTVSS

SEQ ID NO: 39 - protein, 107 aa, Mus musculus
  REGION 1..107: note = M P2-C7 LCVR
DIQMTQSPASLSVSVGETVTITCRTSENIYSNLAWYQQKQGKSPQLLVYGATNLADGVPSRFSGSGSGTQYSLKINSLQSEDFGSYYCQHFWDIPWTFGGGTTLEIK

SEQ ID NO: 40 - protein, 120 aa, Mus musculus
  REGION 1..120: note = M P2-C6 HCVR
EVQLQQSGPELVKPGASVKMSCEASGYTFTDYYIHWVKQSHGESLEWIGYIYPDNGYNGYNQKFKGKATLTVDKSSNTAYMELRSLTSEDSAVYFCTRRGDYSGVHFDYWGQGTALTVSS

SEQ ID NO: 41 - protein, 112 aa, Mus musculus
  REGION 1..112: note = M P2-C6 LCVR
DIVLTQSPASLAVSLGQRATISCRASESVNNYGVGFLHWYQQKPGQPPKLLIYRASTLESGIPARFSGSGSRTDFTLTINPVETDDVATYYCQHSYKDPPWTFGGGTKLEIK

SEQ ID NO: 42 - protein, 120 aa, Mus musculus
  REGION 1..120: note = M P1-D7 HCVR
QIQLVQSGPDLKKPGETVKISCKASGYTFTTYGMNWVKQAPGKALKWMGWINTYSGVPTYADDFKGRFAFSLETSATTAYLQINNLKNEDTATYFCARRTDYDGYVMDCWGQGTSVTVSS

SEQ ID NO: 43 - protein, 113 aa, Mus musculus
  REGION 1..113: note = M P1-D7 LCVR
DIVMSQSPSSLAVSIGEKVTMSCKSSQSLFYSGNQKNYLAWYLQKPGQSPKLLLYWASTRESGVPDRFTGSGSGTDFTLTISSVMAEDLAVYYCQQYFSYPPTFGGGTKLEIK

SEQ ID NO: 44 - protein, 125 aa, Mus musculus
  REGION 1..125: note = M P1-E11 HCVR
EVQLQQSGPELVKPGASVKMSCQASGYTFTDYSIHWVKQSRGASLEWIGYINPNNGVTNYNQKFKGKATLTVNKSSSTAYMELRSLTSEDSAVYYCAREGDSVTTIVVHWYFDVGGTGTTVTVSS

SEQ ID NO: 45 - protein, 107 aa, Mus musculus
  REGION 1..107: note = M P1-E11 LCVR
DIQMTQSPASLSVSLGETVTITCRASENIYSNLVWYQQKQGKFPQLLVYAAINLVDGVPSRFSGSGSGTQYSLKINSLQSEDFGSYYCQQFWDTPLTFGAGTKLEIK

SEQ ID NO: 46 - protein, 123 aa, Mus musculus
  REGION 1..123: note = M P2-B9 HCVR
EVQLQQSGPELVKPGASVKISCKASGYTFTDYFMNWVKLSHGKSLEWIGDINPNNGGTSYNQRFKDKVTLTVDKSSSTAYMELRSLTSDSSAVYFCARNGYYDSNYLSYFDVWGTGTTVTVSS

SEQ ID NO: 47 - protein, 107 aa, Mus musculus
  REGION 1..107: note = M P2-B9 LCVR
DIQMTQSPASLSVSVGETVTITCRASENIYSNLAWYQQKQGKSPQLLVYGATNLADGVPSRFSGSGSGTQYSLKINSLQSEDFGSYYCQHFWDTPYTFGGGTKLEIK

SEQ ID NO: 48 - protein, 117 aa, Mus musculus
  REGION 1..117: note = M P2-C2 HCVR
QVQLKQSGPGLVQPSQSLSITCTVSGFSLTSYGVHWVRQSPGKGLEWLGVIWSGGHTDLNAAFISRLSINKDNSKSQVFFKMNSLQGDDTAIYYCARNGYGGCLDYWGQGTTLTVSS

SEQ ID NO: 49 - protein, 107 aa, Mus musculus
  REGION 1..107: note = M P2-C2 LCVR
DIVMTQSHKFMSTSVGDRVSITCKAGQDVSIAVAWYQQKPGQSPQLLIYSASYRYTGVPDRFTGSGSGTDFTFAISSVQAEDLAVYYCQQYYSIPPSFGAGTKLEIK

SEQ ID NO: 50 - protein, 123 aa, Mus musculus
  REGION 1..123: note = M P2-E10 HCVR
DVQLQESGPGLVKPSQSLSLTCSVTGYSITSGYYWNWIRQFPGNKLEWMGYMSYEGTNNSNPSLKNRISITRDTSKNQFFLKLNSVTTEDTARYYCARERAYYYGTLGAMDYWGQGTSVTVSS

SEQ ID NO: 51 - protein, 107 aa, Mus musculus
  REGION 1..107: note = M P2-E10 LCVR
DIQMTQSPASLSVSVGETVTITCRASENIYSNLAWYQQKQGKSPQLLVYAATNLADGVPSRFSGSGSGTQYSLKINSMQSEDFGSYYCQHFWDTPFTFGSGTKLEIK

SEQ ID NO: 52 - protein, 5 aa, Mus musculus
  REGION 1..5: note = M P1-B4-HCDR1
NYGVH

SEQ ID NO: 53 - protein, 16 aa, Mus musculus
  REGION 1..16: note = M P1-B4-HCDR2
VIWTGGSTDYNAAFIS

SEQ ID NO: 54 - protein, 9 aa, Mus musculus
  REGION 1..9: note = M P1-B4-HCDR3
TTVVTAMDY

SEQ ID NO: 55 - protein, 11 aa, Mus musculus
  REGION 1..11: note = M P1-B4-LCDR1
KASQDVNIAVV

SEQ ID NO: 56 - protein, 7 aa, Mus musculus
  REGION 1..7: note = M P1-B4-LCDR2
AASYRYT

SEQ ID NO: 57 - protein, 9 aa, Mus musculus
  REGION 1..9: note = M P1-B4-LCDR3
QQHYSSPYT

SEQ ID NO: 58 - protein, 5 aa, Mus musculus
  REGION 1..5: note = M P1-B9-HCDR1
SYGVH

SEQ ID NO: 59 - protein, 16 aa, Mus musculus
  REGION 1..16: note = M P1-B9-HCDR2
VIWSGGNTDYNAAFMS

SEQ ID NO: 60 - protein, 9 aa, Mus musculus
  REGION 1..9: note = M P1-B9-HCDR3
PYDVVPFAY

SEQ ID NO: 61 - protein, 11 aa, Mus musculus
  REGION 1..11: note = M P1-B9-LCDR1
KASQDVNIAVA

SEQ ID NO: 62 - protein, 7 aa, Mus musculus
  REGION 1..7: note = M P1-B9-LCDR2
SASYRYT

SEQ ID NO: 63 - protein, 9 aa, Mus musculus
  REGION 1..9: note = M P1-B9-LCDR3
QQHYSIPFT

SEQ ID NO: 64 - protein, 5 aa, Mus musculus
  REGION 1..5: note = M P1-D10-HCDR1
TYGVH

SEQ ID NO: 65 - protein, 16 aa, Mus musculus
  REGION 1..16: note = M P1-D10-HCDR2
VIWSGGNTDSNAAFIS

SEQ ID NO: 66 - protein, 7 aa, Mus musculus
  REGION 1..7: note = M P1-D10-HCDR3
YSYAMDY

SEQ ID NO: 67 - protein, 11 aa, Mus musculus
  REGION 1..11: note = M P1-D10-LCDR1
KASQDVSNGVA

SEQ ID NO: 68 - protein, 9 aa, Mus musculus
  REGION 1..9: note = M P1-D10-LCDR3
QQHYSTPFT

SEQ ID NO: 69 - protein, 5 aa, Mus musculus
  REGION 1..5: note = M P2-E8-HCDR1
DYGIH

SEQ ID NO: 70 - protein, 17 aa, Mus musculus
  REGION 1..17: note = M P2-E8-HCDR2
YISSGSSIINYADTVKG

SEQ ID NO: 71 - protein, 13 aa, Mus musculus
  REGION 1..13: note = M P2-E8-HCDR3
GPNYYGSSYLLVY

SEQ ID NO: 72 - protein, 9 aa, Mus musculus
  REGION 1..9: note = M P2-E8-LCDR3
QQHYNIPWT

SEQ ID NO: 73 - protein, 5 aa, Mus musculus
  REGION 1..5: note = M P2-C10-HCDR1
SYWMH

SEQ ID NO: 74 - protein, 17 aa, Mus musculus
  REGION 1..17: note = M P2-C10-HCDR2
VIHPNSDTTNYNEKFKN

SEQ ID NO: 75 - protein, 11 aa, Mus musculus
  REGION 1..11: note = M P2-C10-HCDR3
RYDYAYYAMDY

SEQ ID NO: 76 - protein, 11 aa, Mus musculus
  REGION 1..11: note = M P2-C10-LCDR1
KASQDVTTAVA

SEQ ID NO: 77 - protein, 9 aa, Mus musculus
  REGION 1..9: note = M P2-C10-LCDR3
QQHYSTSPT

SEQ ID NO: 78 - protein, 5 aa, Mus musculus
  REGION 1..5: note = M P2-F4-HCDR1
DYGMH

SEQ ID NO: 79 - protein, 17 aa, Mus musculus
  REGION 1..17: note = M P2-F4-HCDR2
YISSGSRIIYYADTVKG

SEQ ID NO: 80 - protein, 11 aa, Mus musculus
  REGION 1..11: note = M P2-F4-HCDR3
FYNYAHYTMDY

SEQ ID NO: 81 - protein, 11 aa, Mus musculus
  REGION 1..11: note = M P2-F4-LCDR1
KASQDVSTAVA

SEQ ID NO: 82 - protein, 9 aa, Mus musculus
  REGION 1..9: note = M P2-F4-LCDR3
QHHYSTPPT

SEQ ID NO: 83 - protein, 16 aa, Mus musculus
  REGION 1..16: note = M P2-B3-HCDR2
MIWSGGNTDYNAAFTS

SEQ ID NO: 84 - protein, 9 aa, Mus musculus
  REGION 1..9: note = M P2-B3-HCDR3
GDYGSSSAY

SEQ ID NO: 85 - protein, 11 aa, Mus musculus
  REGION 1..11: note = M P2-B3-LCDR1
KASQDVSIAVA

SEQ ID NO: 86 - protein, 9 aa, Mus musculus
  REGION 1..9: note = M P2-B3-LCDR3
QQHYSNTLT

SEQ ID NO: 87 - protein, 17 aa, Mus musculus
  REGION 1..17: note = M P2-E7-HCDR2
NINPSNGGPNYNENFKT

SEQ ID NO: 88 - protein, 12 aa, Mus musculus
  REGION 1..12: note = M P2-E7-HCDR3
GDYYGGSYLFAY

SEQ ID NO: 89 - protein, 7 aa, Mus musculus
  REGION 1..7: note = M P2-E7-LCDR2
SSSYRYT

SEQ ID NO: 90 - protein, 9 aa, Mus musculus
  REGION 1..9: note = M P2-E7-LCDR3
QQHYTFPYT

SEQ ID NO: 91 - protein, 5 aa, Mus musculus
  REGION 1..5: note = M P2-G4-HCDR1
DYNMH

SEQ ID NO: 92 - protein, 17 aa, Mus musculus
  REGION 1..17: note = M P2-G4-HCDR2
YINPNNGGTTYNQKFKG

SEQ ID NO: 93 - protein, 12 aa, Mus musculus
  REGION 1..12: note = M P2-G4-HCDR3
SEYYGSTFLFAY

SEQ ID NO: 94 - protein, 9 aa, Mus musculus
  REGION 1..9: note = M P2-G4-LCDR3
QQHYSTPWT

SEQ ID NO: 95 - protein, 5 aa, Mus musculus
  REGION 1..5: note = M P2-C4-HCDR1
TYAIG

SEQ ID NO: 96 - protein, 16 aa, Mus musculus
  REGION 1..16: note = M P2-C4-HCDR2
VIWTGGGTSYNSALKS

SEQ ID NO: 97 - protein, 8 aa, Mus musculus
  REGION 1..8: note = M P2-C4-HCDR3
GDYGPFAY

SEQ ID NO: 98 - protein, 7 aa, Mus musculus
  REGION 1..7: note = M P2-C4-LCDR2
SASYRHT

SEQ ID NO: 99 - protein, 5 aa, Mus musculus
  REGION 1..5: note = M P2-E11-HCDR1
DYYIN

SEQ ID NO: 100 - protein, 17 aa, Mus musculus
  REGION 1..17: note = M P2-E11-HCDR2
WIFPGSGSTYYNEKFKG

SEQ ID NO: 101 - protein, 12 aa, Mus musculus
  REGION 1..12: note = M P2-E11-HCDR3
SGTLVAPYAMDY

SEQ ID NO: 102 - protein, 11 aa, Mus musculus
  REGION 1..11: note = M P2-E11-LCDR1
KASQSVSNDVA

SEQ ID NO: 103 - protein, 7 aa, Mus musculus
  REGION 1..7: note = M P2-E11-LCDR2
YTSNRYT

SEQ ID NO: 104 - protein, 9 aa, Mus musculus
  REGION 1..9: note = M P2-E11-LCDR3
QQDYSFPLT

SEQ ID NO: 105 - protein, 6 aa, Mus musculus
  REGION 1..5: note = M P1-F7-LCDR1
SGYYWN

SEQ ID NO: 106 - protein, 16 aa, Mus musculus
  REGION 1..16: note = M P1-F7-HCDR2
YISYDGNNYYNPSLKN

SEQ ID NO: 107 - protein, 13 aa, Mus musculus
  REGION 1..13: note = M P1-F7-HCDR3
EDGSYSDYDGFAY

SEQ ID NO: 108 - protein, 11 aa, Mus musculus
  REGION 1..11: note = M P1-F7-LCDR1
RANENIYSNLA

SEQ ID NO: 109 - protein, 7 aa, Mus musculus
  REGION 1..7: note = M P1-F7-LCDR2
AATNLAD

SEQ ID NO: 110 - protein, 9 aa, Mus musculus
  REGION 1..9: note = M P1-F7-LCDR3
QQFWGTPYT

SEQ ID NO: 111 - protein, 5 aa, Mus musculus
  REGION 1..5: note = M P2-E3-HCDR1
DYYMN

SEQ ID NO: 112 - protein, 17 aa, Mus musculus
  REGION 1..17: note = M P2-E3-HCDR2
DINPNNGGTSYNQKFKG

SEQ ID NO: 113 - protein, 15 aa, Mus musculus
  REGION 1..15: note = M P2-E3-HCDR3
GGVTTVVATYWYFDV

SEQ ID NO: 114 - protein, 11 aa, Mus musculus
  REGION 1..11: note = M P2-E3-LCDR1
RASENIYSNLA

SEQ ID NO: 115 - protein, 7 aa, Mus musculus
  REGION 1..7: note = M P2-E3-LCDR2
AATNVAD

SEQ ID NO: 116 - protein, 9 aa, Mus musculus
  REGION 1..9: note = M P2-E3-LCDR3
QQFWDTPFT

SEQ ID NO: 117 - protein, 16 aa, Mus musculus
  REGION 1..16: note = M P2-F10-HCDR2
YITYDGSNNYNPSLKN

SEQ ID NO: 118 - protein, 13 aa, Mus musculus
  REGION 1..13: note = M P2-F10-HCDR3
EYSYGSTLSWFAY

SEQ ID NO: 119 - protein, 9 aa, Mus musculus
  REGION 1..9: note = M P2-F10-LCDR3
QHFWDTPYT

SEQ ID NO: 120 - protein, 16 aa, Mus musculus
  REGION 1..16: note = M P2-G9-HCDR2
YLSYDGSNNYNPSLKN

SEQ ID NO: 121 - protein, 14 aa, Mus musculus
  REGION 1..14: note = M P2-G9-HCDR3
EGAHYSGTLSWFAY

SEQ ID NO: 122 - protein, 17 aa, Mus musculus
  REGION 1..17: note = M P1-C4-HCDR2
RIYPGNDNTYYNEKFKD

SEQ ID NO: 123 - protein, 13 aa, Mus musculus
  REGION 1..13: note = M P1-C4-HCDR3
SQDGYYEENAMDY

SEQ ID NO: 124 - protein, 9 aa, Mus musculus
  REGION 1..9: note = M P1-C4-LCDR3
QQFWGSPHT

SEQ ID NO: 125 - protein, 16 aa, Mus musculus
  REGION 1..16: note = M P1-G7-HCDR2
YISYDGGNNYNPFLKN

SEQ ID NO: 126 - protein, 13 aa, Mus musculus
  REGION 1..13: note = M P1-G7-HCDR3
EGGSSWEYYGMDY

SEQ ID NO: 127 - protein, 11 aa, Mus musculus
  REGION 1..11: note = M P1-G7-LCDR1
RASENIYRNLA

SEQ ID NO: 128 - protein, 9 aa, Mus musculus
  REGION 1..9: note = M P1-G7-LCDR3
QQFWGSPYT

SEQ ID NO: 129 - protein, 5 aa, Mus musculus
  REGION 1..5: note = M P2-C7-HCDR1
DYSMH

SEQ ID NO: 130 - protein, 17 aa, Mus musculus
  REGION 1..17: note = M P2-C7-HCDR2
YFNPNNGDTIYNQKFKG

SEQ ID NO: 131 - protein, 15 aa, Mus musculus
  REGION 1..15: note = M P2-C7-HCDR3
EDSVSTNAWDGALDY

SEQ ID NO: 132 - protein, 11 aa, Mus musculus
  REGION 1..11: note = M P2-C7-LCDR1
RTSENIYSNLA

SEQ ID NO: 133 - protein, 7 aa, Mus musculus
  REGION 1..7: note = M P2-C7-LCDR2
GATNLAD

SEQ ID NO: 134 - protein, 9 aa, Mus musculus
  REGION 1..9: note = M P2-C7-LCDR3
QHFWDIPWT

SEQ ID NO: 135 - protein, 5 aa, Mus musculus
  REGION 1..5: note = M P2-C6-HCDR1
DYYIH

SEQ ID NO: 136 - protein, 17 aa, Mus musculus
  REGION 1..17: note = M P2-C6-HCDR2
YIYPDNGYNGYNQKFKG

SEQ ID NO: 137 - protein, 11 aa, Mus musculus
  REGION 1..11: note = M P2-C6-HCDR3
RGDYSGVHFDY

SEQ ID NO: 138 - protein, 15 aa, Mus musculus
  REGION 1..15: note = M P2-C6-LCDR1
RASESVNNYGVGFLH

SEQ ID NO: 139 - protein, 7 aa, Mus musculus
  REGION 1..7: note = M P2-C6-LCDR2
RASTLES

SEQ ID NO: 140 - protein, 10 aa, Mus musculus
  REGION 1..10: note = M P2-C6-LCDR3
QHSYKDPPWT

SEQ ID NO: 141 - protein, 5 aa, Mus musculus
  REGION 1..5: note = M P1-D7-HCDR1
TYGMN

SEQ ID NO: 142 - protein, 17 aa, Mus musculus
  REGION 1..17: note = M P1-D7-HCDR2
WINTYSGVPTYADDFKG

SEQ ID NO: 143 - protein, 11 aa, Mus musculus
  REGION 1..11: note = M P1-D7-HCDR3
RTDYDGYVMDC

SEQ ID NO: 144 - protein, 17 aa, Mus musculus
  REGION 1..17: note = M P1-D7-LCDR1
KSSQSLFYSGNQKNYLA

SEQ ID NO: 145 - protein, 7 aa, Mus musculus
  REGION 1..7: note = M P1-D7-LCDR2
WASTRES

SEQ ID NO: 146 - protein, 9 aa, Mus musculus
  REGION 1..9: note = M P1-D7-LCDR3
QQYFSYPPT

SEQ ID NO: 147 - protein, 5 aa, Mus musculus
  REGION 1..5: note = M P1-E11-HCDR1
DYSIH

SEQ ID NO: 148 - protein, 17 aa, Mus musculus
  REGION 1..17: note = M P1-E11-HCDR2
YINPNNGVTNYNQKFKG

SEQ ID NO: 149 - protein, 16 aa, Mus musculus
  REGION 1..16: note = M P1-E11-HCDR3
EGDSVTTIVVHWYFDV

SEQ ID NO: 150 - protein, 11 aa, Mus musculus
  REGION 1..11: note = M P1-E11-LCDR1
RASENIYSNLV

SEQ ID NO: 151 - protein, 7 aa, Mus musculus
  REGION 1..7: note = M P1-E11-LCDR2
AAINLVD

SEQ ID NO: 152 - protein, 9 aa, Mus musculus
  REGION 1..9: note = M P1-E11-LCDR3
QQFWDTPLT

SEQ ID NO: 153 - protein, 5 aa, Mus musculus
  REGION 1..5: note = M P2-B9-HCDR1
DYFMN

SEQ ID NO: 154 - protein, 17 aa, Mus musculus
  REGION 1..17: note = M P2-B9-HCDR2
DINPNNGGTSYNQRFKD

SEQ ID NO: 155 - protein, 14 aa, Mus musculus
  REGION 1..14: note = M P2-B9-HCDR3
NGYYDSNYLSYFDV

SEQ ID NO: 156 - protein, 16 aa, Mus musculus
  REGION 1..16: note = M P2-C2-HCDR2
VIWSGGHTDLNAAFIS

SEQ ID NO: 157 - protein, 9 aa, Mus musculus
  REGION 1..9: note = M P2-C2-HCDR3
NGYGGCLDY

SEQ ID NO: 158 - protein, 11 aa, Mus musculus
  REGION 1..11: note = M P2-C2-LCDR1
KAGQDVSIAVA

SEQ ID NO: 159 - protein, 9 aa, Mus musculus
  REGION 1..9: note = M P2-C2-LCDR3
QQYYSIPPS

SEQ ID NO: 160 - protein, 16 aa, Mus musculus
  REGION 1..16: note = M P2-E10-HCDR2
YMSYEGTNNSNPSLKN

SEQ ID NO: 161 - protein, 14 aa, Mus musculus
  REGION 1..14: note = M P2-E10-HCDR3
ERAYYYGTLGAMDY

SEQ ID NO: 162 - protein, 9 aa, Mus musculus
  REGION 1..9: note = M P2-E10-LCDR3
QHFWDTPFT

SEQ ID NO: 163 - protein, 117 aa, synthetic construct
  source 1..117: note = HCVR
  REGION 1..117: note = P2 HCVR
QVQLVQSGAEVKKPGSSVKVSCKASGYTFTSYDISWVRQAPGQGLEWMGGIIPIFGTANYAQKFQGRVTITADESTSTAYMELSSLRSEDTAVYYCTAGIFLATAYWGQGTLVTVSS

SEQ ID NO: 164 - protein, 107 aa, synthetic construct
  source 1..107: note = LCVR
  REGION 1..107: note = P2 LCVR
DIQMTQSPSSMSASVGDRVTISCQASQDINNYLNWYQQRPGQAPKLLIYDASTLETGVPSRFSGSGSGTYFTLTITSLQPADVATYYCQQYENVPITFGQGTRLEIK

SEQ ID NO: 165 - protein, 5 aa, synthetic construct
  source 1..5: note = CDR
  REGION 1..5: note = P2-HCDR1
SYDIS

SEQ ID NO: 166 - protein, 17 aa, synthetic construct
  source 1..17: note = CDR
  REGION 1..17: note = P2-HCDR2
GIIPIFGTANYAQKFQG

SEQ ID NO: 167 - protein, 8 aa, synthetic construct
  source 1..8: note = CDR
  REGION 1..8: note = P2-HCDR3
GIFLATAY

SEQ ID NO: 168 - protein, 11 aa, synthetic construct
  source 1..11: note = CDR
  REGION 1..11: note = P2-LCDR1
QASQDINNYLN

SEQ ID NO: 169 - protein, 7 aa, synthetic construct
  source 1..7: note = CDR
  REGION 1..7: note = P2-LCDR2
DASTLET

SEQ ID NO: 170 - protein, 9 aa, synthetic construct
  source 1..9: note = CDR
  REGION 1..9: note = P2-LCDR3
QQYENVPIT

SEQ ID NO: 171 - protein, 327 aa, Homo sapiens
  REGION 1..327: note = hIgG4-LALA
ASTKGPSVFPLAPCSRSTSESTAALGCLVKDYFPEPVTVSWNSGALTSGVHTFPAVLQSSGLYSLSSVVTVPSSSLGTKTYTCNVDHKPSNTKVDKRVESKYGPPCPPCPAPEAAGGPSVFLFPPKPKDTLMISRTPEVTCVVVDVSQEDPEVQFNWYVDGVEVHNAKTKPREEQFNSTYRVVSVLTVLHQDWLNGKEYKCKVSNKGLPSSIEKTISKAKGQPREPQVYTLPPSQEEMTKNQVSLTCLVKGFYPSDIAVEWESNGQPENNYKTTPPVLDSDGSFFLYSRLTVDKSRWQEGNVFSCSVMHEALHNHYTQKSLSLSLGK

SEQ ID NO: 172 - protein, 107 aa, Homo sapiens [sequence omitted]

SEQ ID NO: 173 - protein, 17 aa, synthetic construct
  source 1..17: note = CDR
  REGION 1..17: note = huP2-E3 VH3-HCDR2
DINPNSGGTSYNQKFKG

SEQ ID NO: 174 - protein, 17 aa, synthetic construct
  source 1..17: note = CDR
  REGION 1..17: note = huP2-E3 VH4-HCDR2
DINPNTGGTSYNQKFKG

SEQ ID NO: 175 - protein, 17 aa, synthetic construct
  source 1..17: note = CDR
  REGION 1..17: note = huP2-E3 VH5-HCDR2
DINPNNVGTSYNQKFKG

SEQ ID NO: 176 - protein, 124 aa, synthetic construct
  source 1..124: note = variable region
  REGION 1..124: note = huP2-E3 VH1
EVQLVQSGAEVKKPGASVKVSCKASGYTFTDYYMNWVRQAPGQRLEWMGDINPNNGGTSYNQKFKGRVTITVDKSASTAYMELSSLRSEDTAVYYCARGGVTTVVATYWYFDVWGQGTTVTVSS

SEQ ID NO: 177 - protein, 124 aa, synthetic construct
  source 1..124: note = variable region
  REGION 1..124: note = huP2-E3 VH2
EVQLVQSGAEVKKPGASVKVSCKASGYTFTDYYMNWVRQAPGQSLEWMGDINPNNGGTSYNQKFKGRVTLTVDKSASTAYMELSSLRSEDTAVYYCARGGVTTVVATYWYFDVWGQGTTVTVSS

SEQ ID NO: 178 - protein, 124 aa, synthetic construct
  source 1..124: note = variable region
  REGION 1..124: note = huP2-E3 VH3
EVQLVQSGAEVKKPGASVKVSCKASGYTFTDYYMNWVRQAPGQSLEWMGDINPNSGGTSYNQKFKGRVTLTVDKSASTAYMELSSLRSEDTAVYYCARGGVTTVVATYWYFDVWGQGTTVTVSS

SEQ ID NO: 179 - protein, 124 aa, synthetic construct
  source 1..124: note = variable region
  REGION 1..124: note = huP2-E3 VH4
EVQLVQSGAEVKKPGASVKVSCKASGYTFTDYYMNWVRQAPGQSLEWMGDINPNTGGTSYNQKFKGRVTLTVDKSASTAYMELSSLRSEDTAVYYCARGGVTTVVATYWYFDVWGQGTTVTVSS

SEQ ID NO: 180 - protein, 124 aa, synthetic construct
  source 1..124: note = variable region
  REGION 1..124: note = huP2-E3 VH5
EVQLVQSGAEVKKPGASVKVSCKASGYTFTDYYMNWVRQAPGQSLEWMGDINPNNVGTSYNQKFKGRVTLTVDKSASTAYMELSSLRSEDTAVYYCARGGVTTVVATYWYFDVWGQGTTVTVSS

SEQ ID NO: 181 - protein, 124 aa, synthetic construct
  source 1..124: note = variable region
  REGION 1..124: note = huP2-E3 VH6
EVQLVQSGAEVKKPGASVKVSCKASGYTFTDYYMNWVKQAPGQRLEWMGDINPNSGGTSYNQKFKGRVTITVDKSGSTAYMELSSLRSEDTAVYYCARGGVTTVVATYWYFDVWGQGTTVTVSS

SEQ ID NO: 182 - protein, 107 aa, synthetic construct
  source 1..107: note = variable region
  REGION 1..107: note = huP2-E3 VL1
DIQMTQSPSSLSASVGDRVTITCRASENIYSNLAWYQQKPGKAPKLLVYAATNVADGVPSRFSGSGSGTDFTLTISSLQPEDFATYYCQQFWDTPFTFGQGTKLEIK

SEQ ID NO: 183 - protein, 107 aa, synthetic construct
  source 1..107: note = variable region
  REGION 1..107: note = huP2-E3 VL2
DIQMTQSPSSLSASVGDRVTITCRASENIYSNLAWYQQKPGKSPKLLVYAATNVADGVPSRFSGSGSGTDYTLTISSLQPEDFATYYCQQFWDTPFTFGQGTKLEIK

SEQ ID NO: 184 - protein, 123 aa, synthetic construct
  source 1..123: note = variable region
  REGION 1..123: note = huP2-G9 VH1
EVQLQESGPGLVKPSQTLSLTCTVSGSSITSGYYWNWIRQHPGKGLEWIGYLSYDGSNNYNPSLKNLVTISRDTSKNQFSLKLSSVTAADTAVYYCAREGAHYSGTLSWFAYWGQGTLVTVSS

SEQ ID NO: 185 - protein, 123 aa, synthetic construct
  source 1..123: note = variable region
  REGION 1..123: note = huP2-G9 VH2
EVQLQESGPGLVKPSQTLSLTCTVSGSSITSGYYWNWIRQHPGKKLEWIGYLSYDGSNNYNPSLKNLVTISRDTSKSQFSLKLSSVTAADTAVYYCAREGAHYSGTLSWFAYWGQGTLVTVSS

SEQ ID NO: 186 - protein, 107 aa, synthetic construct
  source 1..107: note = variable region
  REGION 1..107: note = huP2-G9 VL1
DIQMTQSPSSLSASVGDRVTITCRASENIYSNLAWYQQKPGKAPKLLVYAATNLADGVPSRFSGSGSGTDFTLTISSLQPEDFATYYCQHFWDTPYTFGGGTKVEIK

SEQ ID NO: 187 - protein, 107 aa, synthetic construct
  source 1..107: note = variable region
  REGION 1..107: note = huP2-G9 VL2
DIQMTQSPSSLSASVGDRVTITCRASENIYSNLAWYQQKPGKSPKLLVYAATNLADGVPSRFSGSGSGTDYTLTISSLQPEDFATYYCQHFWDTPYTFGGGTKVEIK

SEQ ID NO: 188 - protein, 17 aa, synthetic construct
  source 1..17: note = CDR
  REGION 1..17: note = huP2-E8 VH3-HCDR2
YISSGSNIINYADTVKG

SEQ ID NO: 189 - protein, 17 aa, synthetic construct
  source 1..17: note = CDR
  REGION 1..17: note = huP2-E8 VH4-HCDR2
YISSGSSIHNYADTVKG

SEQ ID NO: 190 - protein, 122 aa, synthetic construct
  source 1..122: note = variable region
  REGION 1..122: note = huP2-E8 VH1
EVQLVESGGGLVKPGGSLRLSCAASGFTFSDYGIHWVRQAPGKGLEWVSYISSGSSIINYADTVKGRFTISRDNAKNSLYLQMNSLRAEDTAVYYCARGPNYYGSSYLLVYWGQGTLVTVSS

SEQ ID NO: 191 - protein, 122 aa, synthetic construct
  source 1..122: note = variable region
  REGION 1..122: note = huP2-E8 VH2
EVQLVESGGGLVKPGGSLRLSCAASGFTFSDYGIHWVRQAPGKGLEWVAYISSGSSIINYADTVKGRFTISRDNAKNSLYLQMNSLRAEDTAVYYCARGPNYYGSSYLLVYWGQGTLVTVSS

SEQ ID NO: 192 - protein, 122 aa, synthetic construct
  source 1..122: note = variable region
  REGION 1..122: note = huP2-E8 VH3
EVQLVESGGGLVKPGGSLRLSCAASGFTFSDYGIHWVRQAPGKGLEWVAYISSGSNIINYADTVKGRFTISRDNAKNSLYLQMNSLRAEDTAVYYCARGPNYYGSSYLLVYWGQGTLVTVSS

SEQ ID NO: 193 - protein, 122 aa, synthetic construct
  source 1..122: note = variable region
  REGION 1..122: note = huP2-E8 VH4
EVQLVESGGGLVKPGGSLRLSCAASGFTFSDYGIHWVRQAPGKGLEWVAYISSGSSIHNYADTVKGRFTISRDNAKNSLYLQMNSLRAEDTAVYYCARGPNYYGSSYLLVYWGQGTLVTVSS

SEQ ID NO: 194 - protein, 107 aa, synthetic construct
  source 1..107: note = variable region
  REGION 1..107: note = huP2-E8 VL1
DIQMTQSPSSLSASVGDRVTITCKASQDVNIAVAWYQQKPGKAPKLLIYSASYRYTGVPSRFSGSGSGTDFTFTISSLQPEDIATYYCQQHYNIPWTFGGGTKVEIK

SEQ ID NO: 195 - protein, 107 aa, synthetic construct
  source 1..107: note = variable region
  REGION 1..107: note = huP2-E8 VL2
DIQMTQSPSSLSASVGDRVTITCKASQDVNIAVAWYQQKPGKSPKLLIYSASYRYTGVPSRFSGSGSGTDFTFTISSLQPEDIAVYYCQQHYNIPWTFGGGTKVEIK

SEQ ID NO: 196 - protein, 107 aa, synthetic construct
  source 1..107: note = variable region
  REGION 1..107: note = huP2-E8 VL3
DIQMTQSPSSLSASVGDRVTITCKASQDVNIAVAWYQQRPGQSPKLLIYSASYRYTGVPSRFSGSGSGTDFTFTISSLQPEDIAVYYCQQHYNIPWTFGGGTKVEIK

SEQ ID NO: 197 - protein, 122 aa, synthetic construct
  source 1..122: note = variable region
  REGION 1..122: note = huP1-G7 VH1
EVQLQESGPGLVKPSQTLSLTCTVSGYSITSGYYWNWIRQHPGKGLEWIGYISYDGGNNYNPFLKNRVTISRDTSKNQFSLKLSSVTAADTAVYYCAREGGSSWEYYGMDYWGQGTTVTVSS

SEQ ID NO: 198 - protein, 122 aa, synthetic construct
  source 1..122: note = variable region
  REGION 1..122: note = huP1-G7 VH2
EVQLQESGPGLVKPSQTLSLTCTVSGYSITSGYYWNWIRQHPEKKLEWIGYISYDGGNNYNPFLKNRVTISRDTSKNQFSLKLSSVTAADTAVYYCAREGGSSWEYYGMDYWGQGTTVTVSS

SEQ ID NO: 199 - protein, 107 aa, synthetic construct
  source 1..107: note = variable region
  REGION 1..107: note = huP1-G7 VL1
DIQMTQSPSSLSASVGDRVTITCRASENIYRNLAWYQQKPGKAPKLLLYAATNLADGVPSRFSGSGSGTDFTLTISSLQPEDFATYYCQQFWGSPYTFGGGTKVEIK

SEQ ID NO: 200 - protein, 107 aa, synthetic construct
  source 1..107: note = variable region
  REGION 1..107: note = huP1-G7 VL2
DIQMTQSPSSLSASVGDRVTITCRASENIYRNLAWYQQKPGKSPKLLLYAATNLADGVPSRFSGSGSGTDYTLTISSLQPEDFATYYCQQFWGSPYTFGGGTKVEIK

SEQ ID NO: 201 - protein, 17 aa, synthetic construct
  source 1..17: note = CDR
  REGION 1..17: note = huP2-C6 VH3-HCDR2
YIYPDNGYSGYNQKFKG

SEQ ID NO: 202 - protein, 17 aa, synthetic construct
  source 1..17: note = CDR
  REGION 1..17: note = huP2-C6 VH4-HCDR2
YIYPDNGYTGYNQKFKG

SEQ ID NO: 203 - protein, 17 aa, synthetic construct
  source 1..17: note = CDR
  REGION 1..17: note = huP2-C6 VH5-HCDR2
YIYPDTGYSGYNQKFKG

SEQ ID NO: 204 - protein, 17 aa, synthetic construct
  source 1..17: note = CDR
  REGION 1..17: note = huP2-C6 VH6-HCDR2
YIYPDSGYNGYNQKFKG

SEQ ID NO: 205 - protein, 120 aa, synthetic construct
  source 1..120: note = variable region
  REGION 1..120: note = huP2-C6 VH1
EVQLVQSGAEVKKPGASVKVSCKASGYTFTDYYIHWVRQAPGQGLEWMGYIYPDNGYNGYNQKFKGRVTMTVDKSTSTAYMELRSLRSDDTAVYYCTRRGDYSGVHFDYWGQGTTVTVSS

SEQ ID NO: 206 - protein, 120 aa, synthetic construct
  source 1..120: note = variable region
  REGION 1..120: note = huP2-C6 VH2
EVQLVQSGAEVKKPGASVKVSCKASGYTFTDYYIHWVRQAPGEGLEWMGYIYPDNGYNGYNQKFKGRVTLTVDKSTNTAYMELRSLRSDDTAVYYCTRRGDYSGVHFDYWGQGTTVTVSS

SEQ ID NO: 207 - protein, 120 aa, synthetic construct
  source 1..120: note = variable region
  REGION 1..120: note = huP2-C6 VH3
EVQLVQSGAEVKKPGASVKVSCKASGYTFTDYYIHWVRQAPGEGLEWMGYIYPDNGYSGYNQKFKGRVTLTVDKSTNTAYMELRSLRSDDTAVYYCTRRGDYSGVHFDYWGQGTTVTVSS

SEQ ID NO: 208 - protein, 120 aa, synthetic construct
  source 1..120: note = variable region
  REGION 1..120: note = huP2-C6 VH4
EVQLVQSGAEVKKPGASVKVSCKASGYTFTDYYIHWVRQAPGEGLEWMGYIYPDNGYTGYNQKFKGRVTLTVDKSTNTAYMELRSLRSDDTAVYYCTRRGDYSGVHFDYWGQGTTVTVSS

SEQ ID NO: 209 - protein, 120 aa, synthetic construct
  source 1..120: note = variable region
  REGION 1..120: note = huP2-C6 VH5
EVQLVQSGAEVKKPGASVKVSCKASGYTFTDYYIHWVRQAPGEGLEWMGYIYPDTGYSGYNQKFKGRVTLTVDKSTNTAYMELRSLRSDDTAVYYCTRRGDYSGVHFDYWGQGTTVTVSS

SEQ ID NO: 210 - protein, 120 aa, synthetic construct
  source 1..120: note = variable region
  REGION 1..120: note = huP2-C6 VH6
EVQLVQSGAEVKKPGASVKVSCKASGYTFTDYYIHWVRQAPGEGLEWMGYIYPDSGYNGYNQKFKGRVTLTVDKSTNTAYMELRSLRSDDTAVYYCTRRGDYSGVHFDYWGQGTTVTVSS

SEQ ID NO: 211 - protein, 120 aa, synthetic construct
  source 1..120: note = variable region
  REGION 1..120: note = huP2-C6 VH7
EVQLVQSGAEVKKPGASVKVSCKASGYTFTDYYIHWVRQAPGQGLEWMGYIYPDTGYSGYNQKFKGRVTMTVDKSTSTAYMELRSLRSDDTAVYYCTRRGDYSGVHFDYWGQGTTVTVSS

SEQ ID NO: 212 - protein, 112 aa, synthetic construct
  source 1..112: note = variable region
  REGION 1..112: note = huP2-C6 VL1
DIVLTQSPDSLAVSLGERATINCRASESVNNYGVGFLHWYQQKPGQPPKLLIYRASTLESGIPDRFSGSGSGTDFTLTISSLQAEDVAVYYCQHSYKDPPWTFGGGTKVEIK

SEQ ID NO: 213 - protein, 112 aa, synthetic construct
  source 1..112: note = variable region
  REGION 1..112: note = huP2-C6 VL2
DIVLTQSPDSLAVSLGERATINCRASESVNNYGVGFLHWYQQKPGQPPKLLIYRASTLESGIPDRFSGSGSRTDFTLTISSLQAEDVATYYCQHSYKDPPWTFGGGTKVEIK

SEQ ID NO: 214 - protein, 112 aa, synthetic construct
  source 1..112: note = variable region
  REGION 1..112: note = huP2-C6 VL3
EIVLTQSPATLSLSPGERATLSCRASESVNNYGVGFLHWYQQKPGQPPKLLIYRASTLESGIPARFSGSGSRTDFTLTISSLEPEDFAVYYCQHSYKDPPWTFGGGTKVEIK

SEQ ID NO: 215 - protein, 17 aa, synthetic construct
  source 1..17: note = CDR
  REGION 1..17: note = huP1-D7 VH1-HCDR2
WINTYSGVPTYAEDFKG

SEQ ID NO: 216 - protein, 11 aa, synthetic construct
  source 1..11: note = CDR
  REGION 1..11: note = huP1-D7 VH1-HCDR3
RTDYDGYVMDS

SEQ ID NO: 217 - protein, 120 aa, synthetic construct
  source 1..120: note = variable region
  REGION 1..120: note = huP1-D7 VH1
EVQLVQSGAEVKKPGASVKVSCKASGYTFTTYGMNWVRQAPGQGLEWMGWINTYSGVPTYAEDFKGRVTMTTDTSTSTAYMELRSLRSDDTAVYYCARRTDYDGYVMDSWGQGTTVTVSS

SEQ ID NO: 218 - protein, 120 aa, synthetic construct
  source 1..120: note = variable region
  REGION 1..120: note = huP1-D7 VH2
EIQLVQSGAEVKKPGASVKVSCKASGYTFTTYGMNWVRQAPGQGLEWMGWINTYSGVPTYAEDFKGRVTMTTDTSTTTAYMELRSLRSDDTAVYYCARRTDYDGYVMDSWGQGTTVTVSS

SEQ ID NO: 219 - protein, 120 aa, synthetic construct
  source 1..120: note = variable region
  REGION 1..120: note = huP1-D7 VH3
EIQLVQSGAEVKKPGASVKVSCKASGYTFTTYGMNWVRQAPGQALKWMGWINTYSGVPTYAEDFKGRVTMTTDTSTTTAYMELRSLRSDDTAVYYCARRTDYDGYVMDSWGQGTTVTVSS

SEQ ID NO: 220 - protein, 120 aa, synthetic construct
  source 1..120: note = variable region
  REGION 1..120: note = huP1-D7 VH4
EIQLVQSGAEVKKPGASVKVSCKASGYTFTTYGMNWVRQAPGQALKWMGWINTYSGVPTYADDFKGRVTMTTDTSTTTAYMELRSLRSDDTAVYYCARRTDYDGYVMDSWGQGTTVTVSS

SEQ ID NO: 221 - protein, 120 aa, synthetic construct
  source 1..120: note = variable region
  REGION 1..120: note = huP1-D7 VH5
EIQLVQSGAEVKKPGASVKVSCKASGYTFTTYGMNWVRQAPGQALKWMGWINTYSGVPTYADDFKGRVTMTTDTSTTTAYMELRSLRSDDTAVYYCARRTDYDGYVMDCWGQGTTVTVSS

SEQ ID NO: 222 - protein, 113 aa, synthetic construct
  source 1..113: note = variable region
  REGION 1..113: note = huP1-D7 VL1
DIVMTQSPDSLAVSLGERATINCKSSQSLFYSGNQKNYLAWYQQKPGQSPKLLLYWASTRESGVPDRFSGSGSGTDFTLTISSLQAEDVAVYYCQQYFSYPPTFGGGTKVEIK

SEQ ID NO: 223 - protein, 113 aa, synthetic construct
  source 1..113: note = variable region
  REGION 1..113: note = huP1-D7 VL2
DIVMTQSPLSLPVTPGEPASISCKSSQSLFYSGNQKNYLAWYLQKPGQSPQLLLYWASTRESGVPDRFSGSGSGTDFTLKISRVEAEDVGVYYCQQYFSYPPTFGGGTKVEIK

SEQ ID NO: 224 - protein, 11 aa, synthetic construct
  source 1..11: note = CDR
  REGION 1..11: note = P2-VL1-LCDR1
QASQDIQNYLN

SEQ ID NO: 225 - protein, 107 aa, synthetic construct
  source 1..107: note = variable region
  REGION 1..107: note = P2m LCVR
DIQMTQSPSSMSASVGDRVTISCQASQDIQNYLNWYQQRPGQAPKLLIYDASTLETGVPSRFSGSGSGTYFTLTISSLQPEDVATYYCQQYENVPITFGQGTRLEIK

SEQ ID NO: 226 - protein, 451 aa, synthetic construct
  source 1..451: note = HC
  CHAIN 1..451: note = huP2-E3-heavy chain
EVQLVQSGAEVKKPGASVKVSCKASGYTFTDYYMNWVKQAPGQRLEWMGDINPNSGGTSYNQKFKGRVTITVDKSGSTAYMELSSLRSEDTAVYYCARGGVTTVVATYWYFDVWGQGTTVTVSSASTKGPSVFPLAPCSRSTSESTAALGCLVKDYFPEPVTVSWNSGALTSGVHTFPAVLQSSGLYSLSSVVTVPSSSLGTKTYTCNVDHKPSNTKVDKRVESKYGPPCPPCPAPEAAGGPSVFLFPPKPKDTLMISRTPEVTCVVVDVSQEDPEVQFNWYVDGVEVHNAKTKPREEQFNSTYRVVSVLTVLHQDWLNGKEYKCKVSNKGLPSSIEKTISKAKGQPREPQVYTLPPSQEEMTKNQVSLTCLVKGFYPSDIAVEWESNGQPENNYKTTPPVLDSDGSFFLYSRLTVDKSRWQEGNVFSCSVMHEALHNHYTQKSLSLSLGK

SEQ ID NO: 227 - protein, 214 aa, synthetic construct
  source 1..214: note = LC
  CHAIN 1..214: note = huP2-E3-light chain
DIQMTQSPSSLSASVGDRVTITCRASENIYSNLAWYQQKPGKSPKLLVYAATNVADGVPSRFSGSGSGTDYTLTISSLQPEDFATYYCQQFWDTPFTFGQGTKLEIKRTVAAPSVFIFPPSDEQLKSGTASVVCLLNNFYPREAKVQWKVDNALQSGNSQESVTEQDSKDSTYSLSSTLTLSKADYEKHKVYACEVTHQGLSSPVTKSFNRGEC

SEQ ID NO: 228 - protein, 453 aa, synthetic construct
  source 1..453: note = HC
  REGION 1..453: note = huP2-G9-heavy chain
EVQLQESGPGLVKPSQTLSLTCTVSGSSITSGYYWNWIRQHPGKGLEWIGYLSYDGSNNYNPSLKNLVTISRDTSKNQFSLKLSSVTAADTAVYYCAREGAHYSGTLSWFAYWGQGTLVTVSSASTKGPSVFPLAPSSKSTSGGTAALGCLVKDYFPEPVTVSWNSGALTSGVHTFPAVLQSSGLYSLSSVVTVPSSSLGTQTYICNVNHKPSNTKVDKKVEPKSCDKTHTCPPCPAPEAAGGPSVFLFPPKPKDTLMISRTPEVTCVVVDVSHEDPEVKFNWYVDGVEVHNAKTKPREEQYNSTYRVVSVLTVLHQDWLNGKEYKCKVSNKALPAPIEKTISKAKGQPREPQVYTLPPSRDELTKNQVSLTCLVKGFYPSDIAVEWESNGQPENNYKTTPPVLDSDGSFFLYSKLTVDKSRWQQGNVFSCSVMHEALHNHYTQKSLSLSPGK

SEQ ID NO: 229 - protein, 214 aa, synthetic construct
  source 1..214: note = LC
  CHAIN 1..214: note = huP2-G9-light chain
DIQMTQSPSSLSASVGDRVTITCRASENIYSNLAWYQQKPGKSPKLLVYAATNLADGVPSRFSGSGSGTDYTLTISSLQPEDFATYYCQHFWDTPYTFGGGTKVEIKRTVAAPSVFIFPPSDEQLKSGTASVVCLLNNFYPREAKVQWKVDNALQSGNSQESVTEQDSKDSTYSLSSTLTLSKADYEKHKVYACEVTHQGLSSPVTKSFNRGEC

SEQ ID NO: 230 - protein, 449 aa, synthetic construct
  source 1..449: note = HC
  CHAIN 1..449: note = huP2-E8-heavy chain
EVQLVESGGGLVKPGGSLRLSCAASGFTFSDYGIHWVRQAPGKGLEWVAYISSGSSIHNYADTVKGRFTISRDNAKNSLYLQMNSLRAEDTAVYYCARGPNYYGSSYLLVYWGQGTLVTVSSASTKGPSVFPLAPCSRSTSESTAALGCLVKDYFPEPVTVSWNSGALTSGVHTFPAVLQSSGLYSLSSVVTVPSSSLGTKTYTCNVDHKPSNTKVDKRVESKYGPPCPPCPAPEAAGGPSVFLFPPKPKDTLMISRTPEVTCVVVDVSQEDPEVQFNWYVDGVEVHNAKTKPREEQFNSTYRVVSVLTVLHQDWLNGKEYKCKVSNKGLPSSIEKTISKAKGQPREPQVYTLPPSQEEMTKNQVSLTCLVKGFYPSDIAVEWESNGQPENNYKTTPPVLDSDGSFFLYSRLTVDKSRWQEGNVFSCSVMHEALHNHYTQKSLSLSLGK

SEQ ID NO: 231 - protein, 214 aa, synthetic construct
  source 1..214: note = LC
  CHAIN 1..214: note = huP2-E8-light chain
DIQMTQSPSSLSASVGDRVTITCKASQDVNIAVAWYQQKPGKAPKLLIYSASYRYTGVPSRFSGSGSGTDFTFTISSLQPEDIATYYCQQHYNIPWTFGGGTKVEIKRTVAAPSVFIFPPSDEQLKSGTASVVCLLNNFYPREAKVQWKVDNALQSGNSQESVTEQDSKDSTYSLSSTLTLSKADYEKHKVYACEVTHQGLSSPVTKSFNRGEC

SEQ ID NO: 232 - protein, 449 aa, synthetic construct
  source 1..449: note = HC
  CHAIN 1..449: note = huP1-G7-heavy chain
EVQLQESGPGLVKPSQTLSLTCTVSGYSITSGYYWNWIRQHPGKGLEWIGYISYDGGNNYNPFLKNRVTISRDTSKNQFSLKLSSVTAADTAVYYCAREGGSSWEYYGMDYWGQGTTVTVSSASTKGPSVFPLAPCSRSTSESTAALGCLVKDYFPEPVTVSWNSGALTSGVHTFPAVLQSSGLYSLSSVVTVPSSSLGTKTYTCNVDHKPSNTKVDKRVESKYGPPCPPCPAPEAAGGPSVFLFPPKPKDTLMISRTPEVTCVVVDVSQEDPEVQFNWYVDGVEVHNAKTKPREEQFNSTYRVVSVLTVLHQDWLNGKEYKCKVSNKGLPSSIEKTISKAKGQPREPQVYTLPPSQEEMTKNQVSLTCLVKGFYPSDIAVEWESNGQPENNYKTTPPVLDSDGSFFLYSRLTVDKSRWQEGNVFSCSVMHEALHNHYTQKSLSLSLGK

SEQ ID NO: 233 - protein, 214 aa, synthetic construct
  source 1..214: note = LC
  CHAIN 1..214: note = huP1-G7-light chain
DIQMTQSPSSLSASVGDRVTITCRASENIYRNLAWYQQKPGKAPKLLLYAATNLADGVPSRFSGSGSGTDFTLTISSLQPEDFATYYCQQFWGSPYTFGGGTKVEIKRTVAAPSVFIFPPSDEQLKSGTASVVCLLNNFYPREAKVQWKVDNALQSGNSQESVTEQDSKDSTYSLSSTLTLSKADYEKHKVYACEVTHQGLSSPVTKSFNRGEC

SEQ ID NO: 234 - protein, 450 aa, synthetic construct
  source 1..450: note = HC
  CHAIN 1..450: note = huP2-C6-heavy chain
EVQLVQSGAEVKKPGASVKVSCKASGYTFTDYYIHWVRQAPGQGLEWMGYIYPDTGYSGYNQKFKGRVTMTVDKSTSTAYMELRSLRSDDTAVYYCTRRGDYSGVHFDYWGQGTTVTVSSASTKGPSVFPLAPSSKSTSGGTAALGCLVKDYFPEPVTVSWNSGALTSGVHTFPAVLQSSGLYSLSSVVTVPSSSLGTQTYICNVNHKPSNTKVDKKVEPKSCDKTHTCPPCPAPEAAGGPSVFLFPPKPKDTLMISRTPEVTCVVVDVSHEDPEVKFNWYVDGVEVHNAKTKPREEQYNSTYRVVSVLTVLHQDWLNGKEYKCKVSNKALPAPIEKTISKAKGQPREPQVYTLPPSRDELTKNQVSLTCLVKGFYPSDIAVEWESNGQPENNYKTTPPVLDSDGSFFLYSKLTVDKSRWQQGNVFSCSVMHEALHNHYTQKSLSLSPGK

SEQ ID NO: 235 - protein, 219 aa, synthetic construct
  source 1..219: note = LC
  CHAIN 1..219: note = huP2-C6-light chain
DIVLTQSPDSLAVSLGERATINCRASESVNNYGVGFLHWYQQKPGQPPKLLIYRASTLESGIPDRFSGSGSGTDFTLTISSLQAEDVAVYYCQHSYKDPPWTFGGGTKVEIKRTVAAPSVFIFPPSDEQLKSGTASVVCLLNNFYPREAKVQWKVDNALQSGNSQESVTEQDSKDSTYSLSSTLTLSKADYEKHKVYACEVTHQGLSSPVTKSFNRGEC

SEQ ID NO: 236 - protein, 447 aa, synthetic construct
  source 1..447: note = HC
  CHAIN 1..447: note = huP1-D7-heavy chain
EVQLVQSGAEVKKPGASVKVSCKASGYTFTTYGMNWVRQAPGQGLEWMGWINTYSGVPTYAEDFKGRVTMTTDTSTSTAYMELRSLRSDDTAVYYCARRTDYDGYVMDSWGQGTTVTVSSASTKGPSVFPLAPCSRSTSESTAALGCLVKDYFPEPVTVSWNSGALTSGVHTFPAVLQSSGLYSLSSVVTVPSSSLGTKTYTCNVDHKPSNTKVDKRVESKYGPPCPPCPAPEAAGGPSVFLFPPKPKDTLMISRTPEVTCVVVDVSQEDPEVQFNWYVDGVEVHNAKTKPREEQFNSTYRVVSVLTVLHQDWLNGKEYKCKVSNKGLPSSIEKTISKAKGQPREPQVYTLPPSQEEMTKNQVSLTCLVKGFYPSDIAVEWESNGQPENNYKTTPPVLDSDGSFFLYSRLTVDKSRWQEGNVFSCSVMHEALHNHYTQKSLSLSLGK

SEQ ID NO: 237 - protein, 220 aa, synthetic construct
  source 1..220: note = LC
  CHAIN 1..220: note = huP1-D7-light chain
DIVMTQSPDSLAVSLGERATINCKSSQSLFYSGNQKNYLAWYQQKPGQSPKLLLYWASTRESGVPDRFSGSGSGTDFTLTISSLQAEDVAVYYCQQYFSYPPTFGGGTKVEIKRTVAAPSVFIFPPSDEQLKSGTASVVCLLNNFYPREAKVQWKVDNALQSGNSQESVTEQDSKDSTYSLSSTLTLSKADYEKHKVYACEVTHQGLSSPVTKSFNRGEC

SEQ ID NO: 238 - protein, 447 aa, synthetic construct
  source 1..447: note = HC
  CHAIN 1..447: note = P2m-heavy chain
QVQLVQSGAEVKKPGSSVKVSCKASGYTFTSYDISWVRQAPGQGLEWMGGIIPIFGTANYAQKFQGRVTITADESTSTAYMELSSLRSEDTAVYYCTAGIFLATAYWGQGTLVTVSSASTKGPSVFPLAPSSKSTSGGTAALGCLVKDYFPEPVTVSWNSGALTSGVHTFPAVLQSSGLYSLSSVVTVPSSSLGTQTYICNVNHKPSNTKVDKKVEPKSCDKTHTCPPCPAPEAAGGPSVFLFPPKPKDTLMISRTPEVTCVVVDVSHEDPEVKFNWYVDGVEVHNAKTKPREEQYNSTYRVVSVLTVLHQDWLNGKEYKCKVSNKALPAPIEKTISKAKGQPREPQVYTLPPSRDELTKNQVSLTCLVKGFYPSDIAVEWESNGQPENNYKTTPPVLDSDGSFFLYSKLTVDKSRWQQGNVFSCSVMHEALHNHYTQKSLSLSPGK

SEQ ID NO: 239 - protein, 214 aa, synthetic construct
  source 1..214: note = LC
  CHAIN 1..214: note = P2m-light chain
DIQMTQSPSSMSASVGDRVTISCQASQDIQNYLNWYQQRPGQAPKLLIYDASTLETGVPSRFSGSGSGTYFTLTISSLQPEDVATYYCQQYENVPITFGQGTRLEIKRTVAAPSVFIFPPSDEQLKSGTASVVCLLNNFYPREAKVQWKVDNALQSGNSQESVTEQDSKDSTYSLSSTLTLSKADYEKHKVYACEVTHQGLSSPVTKSFNRGEC

SEQ ID NO: 240 - protein, 330 aa, Homo sapiens
  REGION 1..330: note = hIgG1-LALA
ASTKGPSVFPLAPSSKSTSGGTAALGCLVKDYFPEPVTVSWNSGALTSGVHTFPAVLQSSGLYSLSSVVTVPSSSLGTQTYICNVNHKPSNTKVDKKVEPKSCDKTHTCPPCPAPEAAGGPSVFLFPPKPKDTLMISRTPEVTCVVVDVSHEDPEVKFNWYVDGVEVHNAKTKPREEQYNSTYRVVSVLTVLHQDWLNGKEYKCKVSNKALPAPIEKTISKAKGQPREPQVYTLPPSRDELTKNQVSLTCLVKGFYPSDIAVEWESNGQPENNYKTTPPVLDSDGSFFLYSKLTVDKSRWQQGNVFSCSVMHEALHNHYTQKSLSLSPGK

SEQ ID NO: 241 - protein, 448 aa, synthetic construct
  source 1..448: note = HC
  CHAIN 1..448: note = MK-heavy chain
EVQLQQWGAGLLKPSETLSLTCAVYGGSFSGYYWSWIRQPPGKGLEWIGEINHAGSTNYNPSLKSRVTISVDTSKNQFSLKLSSVTAADTAVYYCARLPTRWVTTRYFDLWGRGTLVTVSSASTKGPSVFPLAPCSRSTSESTAALGCLVKDYFPEPVTVSWNSGALTSGVHTFPAVLQSSGLYSLSSVVTVPSSSLGTKTYTCNVDHKPSNTKVDKRVESKYGPPCPPCPAPEFLGGPSVFLFPPKPKDTLMISRTPEVTCVVVDVSQEDPEVQFNWYVDGVEVHNAKTKPREEQFNSTYRVVSVLTVLHQDWLNGKEYKCKVSNKGLPSSIEKTISKAKGQPREPQVYTLPPSQEEMTKNQVSLTCLVKGFYPSDIAVEWESNGQPENNYKTTPPVLDSDGSFFLYSRLTVDKSRWQEGNVFSCSVMHEALHNHYTQKSLSLSLGK

SEQ ID NO: 242 - protein, 217 aa, synthetic construct
  source 1..217: note = LC
  CHAIN 1..217: note = MK-light chain
ESVLTQPPSVSGAPGQRVTISCTGSSSNIGAGYDVHWYQQLPGTAPKLLIYGDSNRPSGVPDRFSVSKSGASASLAITGLQAEDEADYYCQSFDNSLSAYVFGGGTQLTVLGQPKANPTVTLFPPSSEELQANKATLVCLISDFYPGAVTVAWKADGSPVKAGVETTKPSKQSNNKYAASSYLSLTPEQWKSHRSYSCQVTHEGSTVEKTVAPTECS

SEQ ID NO: 243 - protein, 450 aa, synthetic construct
  source 1..450: note = HC
  CHAIN 1..450: note = JTX-heavy chain
QITLKESGPTLVKPTQTLTLTCTFSGFSLNTYAMGVSWIRQPPGKALEWLASIWWNGNKYNNPSLKSRLTVTKDTSKNQVVLTMTNMDPVDTATYYCAHSRIIRFTDYVMDAWGQGTLVTVSSASTKGPSVFPLAPCSRSTSESTAALGCLVKDYFPEPVTVSWNSGALTSGVHTFPAVLQSSGLYSLSSVVTVPSSSLGTKTYTCNVDHKPSNTKVDKRVESKYGPPCPPCPAPEFLGGPSVFLFPPKPKDTLMISRTPEVTCVVVDVSQEDPEVQFNWYVDGVEVHNAKTKPREEQFNSTYRVVSVLTVLHQDWLNGKEYKCKVSNKGLPSSIEKTISKAKGQPREPQVYTLPPSQEEMTKNQVSLTCLVKGFYPSDIAVEWESNGQPENNYKTTPPVLDSDGSFFLYSRLTVDKSRWQEGNVFSCSVMHEALHNHYTQKSLSLSLGK

SEQ ID NO: 244 - protein, 214 aa, synthetic construct
  source 1..214: note = LC
  CHAIN 1..214: note = JTX-light chain
DIQMTQSPSSLSTSVGDRVTITCRASEDIYNDLAWYQQKPGKAPKLLIYNANSLHTGVASRFSGSGSGTDFTFTISSLQPEDVATYFCQQYYDYPLTFGQGTKLEIKRTVAAPSVFIFPPSDEQLKSGTASVVCLLNNFYPREAKVQWKVDNALQSGNSQESVTEQDSKDSTYSLSSTLTLSKADYEKHKVYACEVTHQGLSSPVTKSFNRGEC

SEQ ID NO: 245 - protein, 444 aa, synthetic construct
  source 1..444: note = ILT2-His
  CHAIN 1..444: note = ILT2-His
GHLPKPTLWAEPGSVITQGSPVTLRCQGGQETQEYRLYREKKTALWITRIPQELVKKGQFPIPSITWEHAGRYRCYYGSDTAGRSESSDPLELVVTGAYIKPTLSAQPSPVVNSGGNVILQCDSQVAFDGFSLCKEGEDEHPQCLNSQPHARGSSRAIFSVGPVSPSRRWWYRCYAYDSNSPYEWSLPSDLLELLVLGVSKKPSLSVQPGPIVAPEETLTLQCGSDAGYNRFVLYKDGERDFLQLAGAQPQAGLSQANFTLGPVSRSYGGQYRCYGAHNLSSEWSAPSDPLDILIAGQFYDRVSLSVQPGPTVASGENVTLLCQSQGWMQTFLLTKEGAADDPWRLRSTYQSQKYQAEFPMGPVTSAHAGTYRCYGSQSSKPYLLTHPSDPLELVVSGPSGGPSSPTTGPTSTSGPEDQPLTPTGSDPQSGLGRHLGVHHHHHH

SEQ ID NO: 246 - protein, 244 aa, synthetic construct
  source 1..244: note = ILT3-His
  CHAIN 1..244: note = ILT3-His
QAGPLPKPTLWAEPGSVISWGNSVTIWCQGTLEAREYRLDKEESPAPWDRQNPLEPKNKARFSIPSMTEDYAGRYRCYYRSPVGWSQPSDPLELVMTGAYSKPTLSALPSPLVTSGKSVTLLCQSRSPMDTFLLIKERAAHPLLHLRSEHGAQQHQAEFPMSPVTSVHGGTYRCFSSHGFSHYLLSHPSDPLELIVSGSLEDPRPSPTRSVSTAAGPEDQPLMPTGSVPHSGLRRHWEHHHHHH

SEQ ID NO: 247 - protein, 338 aa, Homo sapiens
  CHAIN 1..338: note = HLA-G
MVVMAPRTLFLLLSGALTLTETWAGSHSMRYFSAAVSRPGRGEPRFIAMGYVDDTQFVRFDSDSACPRMEPRAPWVEQEGPEYWEEETRNTKAHAQTDRMNLQTLRGYYNQSEASSHTLQWMIGCDLGSDGRLLRGYEQYAYDGKDYLALNEDLRSWTAADTAAQISKRKCEAANVAEQRRAYLEGTCVEWLHRYLENGKEMLQRADPPKTHVTHHPVFDYEATLRCWALGFYPAEIILTWQRDGEDQTQDVELVETRPAGDGTFQKWAAVVVPSGEEQRYTCHVQHEGLPEPLMLRWKQSSLPTIPIMGIVAGLVVLAAVVTGAAVAAVLWRKKSSD

SEQ ID NO: 248 - protein, 452 aa, synthetic construct
  source 1..452: note = HC
  CHAIN 1..452: note = Hu23-11.IgG4AA
EVQLVQSGAEVKKPGSSVKVSCKASGGTFSDYEMHWVRQAPGQGLEWMGLIDPETGGTVYNQKFKDRVTITADKSTSTAYMELSSLRSEDTAVYYCARERFSYYGSTSDWYFDVWGQGTTVTVSSASTKGPSVFPLAPCSRSTSESTAALGCLVKDYFPEPVTVSWNSGALTSGVHTFPAVLQSSGLYSLSSVVTVPSSSLGTKTYTCNVDHKPSNTKVDKRVESKYGPPCPPCPAPEAAGGPSVFLFPPKPKDTLMISRTPEVTCVVVDVSQEDPEVQFNWYVDGVEVHNAKTKPREEQFNSTYRVVSVLTVLHQDWLNGKEYKCKVSNKGLPSSIEKTISKAKGQPREPQVYTLPPSQEEMTKNQVSLTCLVKGFYPSDIAVEWESNGQPENNYKTTPPVLDSDGSFFLYSRLTVDKSRWQEGNVFSCSVMHEALHNHYTQKSLSLSLGK

SEQ ID NO: 249 - protein, 219 aa, synthetic construct
  source 1..219: note = LC
  CHAIN 1..219: note = Hu23-11-light chain
DIVMTQTPLSLPVTPGEPASISCRSSQSLVHSTGNTYLEWYLQKPGQSPQLLIYKVSNRFSGVPDRFSGSGSGTDFTLKISRVEAEDVGVYYCFQGSHVPYTFGGGTKVEIKRTVAAPSVFIFPPSDEQLKSGTASVVCLLNNFYPREAKVQWKVDNALQSGNSQESVTEQDSKDSTYSLSSTLTLSKADYEKHKVYACEVTHQGLSSPVTKSFNRGEC

SEQ ID NO: 250 - protein, 5 aa, synthetic construct
  source 1..5: note = CDR
  REGION 1..5: note = PD-1-HCDR1
DYEMH

SEQ ID NO: 251 - protein, 17 aa, synthetic construct
  source 1..17: note = CDR
  REGION 1..17: note = PD-1-HCDR2
LIDPETGGTVYNQKFKD

SEQ ID NO: 252 - protein, 16 aa, synthetic construct
  source 1..16: note = CDR
  CHAIN 1..16: note = PD-1-HCDR3
ERFSYYGSTSDWYFDV

SEQ ID NO: 253 - protein, 16 aa, synthetic construct
  source 1..16: note = CDR
  REGION 1..16: note = PD-1-LCDR1
RSSQSLVHSTGNTYLE

SEQ ID NO: 254 - protein, 7 aa, synthetic construct
  source 1..7: note = CDR
  CHAIN 1..7: note = PD-1-LCDR2
KVSNRFS

SEQ ID NO: 255 - protein, 9 aa, synthetic construct
  source 1..9: note = CDR
  REGION 1..9: note = PD-1-LCDR3
FQGSHVPYT

SEQ ID NO: 256 - protein, 125 aa, synthetic construct
  source 1..125: note = VH
  REGION 1..125: note = PD-1 VH
EVQLVQSGAEVKKPGSSVKVSCKASGGTFSDYEMHWVRQAPGQGLEWMGLIDPETGGTVYNQKFKDRVTITADKSTSTAYMELSSLRSEDTAVYYCARERFSYYGSTSDWYFDVWGQGTTVTVSS

SEQ ID NO: 257 - protein, 112 aa, synthetic construct
  source 1..112: note = VL
  REGION 1..112: note = PD-1 VL
DIVMTQTPLSLPVTPGEPASISCRSSQSLVHSTGNTYLEWYLQKPGQSPQLLIYKVSNRFSGVPDRFSGSGSGTDFTLKISRVEAEDVGVYYCFQGSHVPYTFGGGTKVEIK

SEQ ID NO: 258 - protein, 448 aa, synthetic construct
  source 1..448: note = HC
  CHAIN 1..448: note = anti PD-1-heavy chain
EVRLLESGGGLVKPEGSLKLSCVASGFTFSDYFMSWVRQAPGKGLEWVAHIYTKSYNYATYYSGSVKGRFTISRDDSRSMVYLQMNNLRTEDTATYYCTRDGSGYPSLDFWGQGTQVTVSSASTKGPSVFPLAPCSRSTSESTAALGCLVKDYFPEPVTVSWNSGALTSGVHTFPAVLQSSGLYSLSSVVTVPSSSLGTKTYTCNVDHKPSNTKVDKRVESKYGPPCPPCPAPEFLGGPSVFLFPPKPKDTLMISRTPEVTCVVVDVSQEDPEVQFNWYVDGVEVHNAKTKPREEQFNSTYRVVSVLTVLHQDWLNGKEYKCKVSNKGLPSSIEKTISKAKGQPREPQVYTLPPSQEEMTKNQVSLTCLVKGFYPSDIAVEWESNGQPENNYKTTPPVLDSDGSFFLYSRLTVDKSRWQEGNVFSCSVMHEALHNHYTQKSLSLSLGK

SEQ ID NO: 259 - protein, 216 aa, synthetic construct
  source 1..216: note = LC
  CHAIN 1..216: note = anti PD-1-light chain
YELTQPPSASVNVGETVKITCSGDQLPKYFADWFHQRSDQTILQVIYDDNKRPSGIPERISGSSSGTTATLTIRDVRAEDEGDYYCFSGYVDSDSKLYVFGSGTQLTVLRTVAAPSVFIFPPSDEQLKSGTASVVCLLNNFYPREAKVQWKVDNALQSGNSQESVTEQDSKDSTYSLSSTLTLSKADYEKHKVYACEVTHQGLSSPVTKSFNRGEC

SEQ ID NO: 260 - protein, 9 aa, Mus musculus
  DOMAIN 1..9: note = huP2-G9-HCDR1-IMGT
GSSITSGYY

SEQ ID NO: 261 - protein, 7 aa, Mus musculus
  DOMAIN 1..7: note = huP2-G9-HCDR2-IMGT
LSYDGSN

SEQ ID NO: 262 - protein, 16 aa, Mus musculus
  DOMAIN 1..16: note = huP2-G9-HCDR3-IMGT
AREGAHYSGTLSWFAY

SEQ ID NO: 263 - protein, 6 aa, Mus musculus
  DOMAIN 1..6: note = huP2-G9-LCDR1-IMGT
ENIYSN

SEQ ID NO: 264 - skipped

SEQ ID NO: 265 - protein, 8 aa, Mus musculus
  DOMAIN 1..8: note = huP2-G9-HCDR1-Chothia
GSSITSGY

SEQ ID NO: 266 - protein, 5 aa, Mus musculus
  DOMAIN 1..5: note = huP2-G9-HCDR2-Chothia
SYDGS

SEQ ID NO: 267 - protein, 8 aa, Mus musculus
  DOMAIN 1..8: note = huP2-C6-HCDR1-IMGT
GYTFTDYY

SEQ ID NO: 268 - protein, 8 aa, synthetic construct
  DOMAIN 1..8: note = huP2-C6-HCDR2-IMGT
IYPDTGYS

SEQ ID NO: 269 - protein, 13 aa, Mus musculus
  DOMAIN 1..13: note = huP2-C6-HCDR3-IMGT
TRRGDYSGVHFDY

SEQ ID NO: 270 - protein, 10 aa, Mus musculus
  DOMAIN 1..10: note = huP2-C6-LCDR1-IMGT
ESVNNYGVGF

SEQ ID NO: 271 - skipped

SEQ ID NO: 272 - protein, 7 aa, Mus musculus
  DOMAIN 1..7: note = huP2-C6-HCDR1-Chothia
GYTFTDY

SEQ ID NO: 273 - protein, 6 aa, synthetic construct
  DOMAIN 1..6: note = huP2-C6-HCDR2-Chothia
YPDTGY